European Patent Application EP 4 800 032 A1, published September 2, 2026. Title: 基于T细胞受体的多特异性多肽分子及其组合物和用途. Applicant: 北京可瑞生物科技有限公司. The sequence listing filed with the application follows.

SEQUENCE LISTING (166 sequences)

SEQ ID NO: 1 - protein, 4 aa, synthetic construct
  REGION 1..4: note = Human IgG1 core hinge region
CPPC

SEQ ID NO: 2 - protein, 609 aa, Homo sapiens [sequence omitted]

SEQ ID NO: 3 - protein, 20 aa, synthetic construct
  REGION 1..20: note = Albumin-binding peptide
QRLMEDICLPRWGCLWEDDF

SEQ ID NO: 4 - protein, 20 aa, synthetic construct
  REGION 1..20: note = Hinge region
EPKSSDKTHTCPPCPAPPVA

SEQ ID NO: 5 - protein, 104 aa, synthetic construct
  REGION 1..104: note = CH2
GPSVFLFPPKPKDTLMISRTPEVTCVVVDVSHEDPEVKFNWYVDGVEVHNAKTKPREEQYQSTYRVVSVLTVLHQDWLNGKEYKCKVSNKGLPSSIEKTISKAK

SEQ ID NO: 6 - protein, 107 aa, synthetic construct
  REGION 1..107: note = CH3 Hole
GQPREPQVCTLPPSRDELTKNQVSLSCAVKGFYPSDIAVEWESNGQPENNYKTTPPVLDSDGSFFLVSKLTVDKSRWQQGNVFSCSVMHEALHNHYTQKSLSLSPGK

SEQ ID NO: 7 - protein, 107 aa, synthetic construct
  REGION 1..107: note = CH3 Knob
GQPREPQVYTLPPCRDELTKNQVSLWCLVKGFYPSDIAVEWESNGQPENNYKTTPPVLDSDGSFFLYSKLTVDKSRWQQGNVFSCSVMHEALHNHYTQKSLSLSPGK

SEQ ID NO: 8 - protein, 86 aa, synthetic construct
  REGION 1..86: note = TRAC
NIQKPDPAVYQLRDSKSSDKSVCLFTDFDSQTNVSQSKDSDVYITDKCVLDMRSMDFKSNSAVAWSNKSDFACANAFNNSIIPEDT

SEQ ID NO: 9 - protein, 90 aa, synthetic construct
  REGION 1..90: note = TRAC
NIQKPDPAVYQLRDSKSSDKSVCLFTDFDSQTNVSQSKDSDVYITDKCVLDMRSMDFKSNSAVAWSNKSDFACANAFNNSIIPEDTFFPS

SEQ ID NO: 10 - protein, 94 aa, synthetic construct
  REGION 1..94: note = TRAC
NIQKPDPAVYQLRDSKSSDKSVCLFTDFDSQTNVSQSKDSDVYITDKCVLDMRSMDFKSNSAVAWSNKSDFACANAFNNSIIPEDTFFPSPESS

SEQ ID NO: 11 - protein, 130 aa, synthetic construct
  REGION 1..130: note = TRBC2
EDLKNVFPPEVAVFEPSEAEISHTQKATLVCLATGFYPDHVELSWWVNGKEVHSGVCTDPQPLKEQPALNDSRYALSSRLRVSATFWQDPRNHFRCQVQFYGLSENDEWTQDRAKPVTQIVSAEAWGRAD

SEQ ID NO: 12 - protein, 112 aa, synthetic construct
  REGION 1..112: note = TRBC2
EDLKNVFPPEVAVFEPSEAEISHTQKATLVCLATGFYPDHVELSWWVNGKEVHSGVCTDPQPLKEQPALNDSRYALSSRLRVSATFWQDPRNHFRCQVQFQIVSAEAWGRAD

SEQ ID NO: 13 - protein, 130 aa, synthetic construct
  REGION 1..130: note = TRBC1
EDLNKVFPPEVAVFEPSEAEISHTQKATLVCLATGFFPDHVELSWWVNGKEVHSGVCTDPQPLKEQPALNDSRYALSSRLRVSATFWQDPRNHFRCQVQFYGLSENDEWTQDRAKPVTQIVSAEAWGRAD

SEQ ID NO: 14 - protein, 112 aa, synthetic construct
  REGION 1..112: note = TRBC1
EDLNKVFPPEVAVFEPSEAEISHTQKATLVCLATGFFPDHVELSWWVNGKEVHSGVCTDPQPLKEQPALNDSRYALSSRLRVSATFWQDPRNHFRCQVQFQIVSAEAWGRAD

SEQ ID NO: 15 - protein, 107 aa, synthetic construct
  REGION 1..107: note = CL
RADAAPTVSIFPPSSEQLTSGGASVVCFLNNFYPKDINVKWKIDGSERQNGVLNSWTDQDSKDSTYSMSSTLTLTKDEYERHNSYTCEATHKTSTSPIVKSFNRNEC

SEQ ID NO: 16 - protein, 104 aa, synthetic construct
  REGION 1..104: note = CL
RADAAPTVSIFPPSSEQLTSGGASVVCFLNNFYPKDINVKWKIDGSERQNGVLNSWTDQDSKDSTYSMSSTLTLTKDEYERHNSYTCEATHKTSTSPIVKSFNR

SEQ ID NO: 17 - protein, 102 aa, synthetic construct
  REGION 1..102: note = CH1
AKTTPPSVYPLAPGSAAQTNSMVTLGCLVKGYFPEPVTVTWNSGSLSSGVHTFPAVLQSDLYTLSSSVTVPSSPRPSETVTCNVAHPASSTKVDKKIVPRDC

SEQ ID NO: 18 - protein, 97 aa, synthetic construct
  REGION 1..97: note = CH1
AKTTPPSVYPLAPGSAAQTNSMVTLGCLVKGYFPEPVTVTWNSGSLSSGVHTFPAVLQSDLYTLSSSVTVPSSPRPSETVTCNVAHPASSTKVDKKI

SEQ ID NO: 19-20 - skipped (2 entries)

SEQ ID NO: 21 - protein, 4 aa, synthetic construct
  REGION 1..4: note = Linker
GGGS

SEQ ID NO: 22 - protein, 5 aa, synthetic construct
  REGION 1..5: note = Linker
GGGGS

SEQ ID NO: 23 - protein, 8 aa, synthetic construct
  REGION 1..8: note = Linker
GGGSGGGG

SEQ ID NO: 24 - protein, 6 aa, synthetic construct
  REGION 1..6: note = Linker
GGSGGS

SEQ ID NO: 25 - protein, 9 aa, synthetic construct
  REGION 1..9: note = Linker
GGSGGSGGS

SEQ ID NO: 26 - protein, 10 aa, synthetic construct
  REGION 1..10: note = Linker
GGGGSGGGGS

SEQ ID NO: 27 - protein, 15 aa, synthetic construct
  REGION 1..15: note = Linker
GGGGSGGGGSGGGGS

SEQ ID NO: 28 - protein, 24 aa, synthetic construct
  REGION 1..24: note = Linker
GGGGSGGGGSGGGGSGGGGSGGGS

SEQ ID NO: 29 - protein, 30 aa, synthetic construct
  REGION 1..30: note = Linker
GGGGSGGGGSGGGGSGGGGSGGGGSGGGGS

SEQ ID NO: 30 - protein, 7 aa, synthetic construct
  REGION 1..7: note = Linker
GQPKAAP

SEQ ID NO: 31 - protein, 5 aa, synthetic construct
  REGION 1..5: note = Linker
TVLRT

SEQ ID NO: 32 - protein, 6 aa, synthetic construct
  REGION 1..6: note = Linker
TVSSAS

SEQ ID NO: 33 - protein, 5 aa, synthetic construct
  REGION 1..5: note = Linker
GGEGG

SEQ ID NO: 34 - protein, 7 aa, synthetic construct
  REGION 1..7: note = Linker
GSEGGGS

SEQ ID NO: 35 - protein, 29 aa, synthetic construct
  REGION 1..29: note = Linker
RTSGPGDGGKGGPGKGPGGEGTKGTGPGG

SEQ ID NO: 36 - protein, 16 aa, synthetic construct
  REGION 1..16: note = Linker
GKGPGGEGTKGTGPGG

SEQ ID NO: 37 - protein, 7 aa, synthetic construct
  REGION 1..7: note = Linker
TVLSSAS

SEQ ID NO: 38 - protein, 5 aa, synthetic construct
  REGION 1..5: note = Linker
EDLKN

SEQ ID NO: 39 - protein, 5 aa, synthetic construct
  REGION 1..5: note = Linker
EDLNK

SEQ ID NO: 40 - protein, 5 aa, synthetic construct
  REGION 1..5: note = Linker
ANIQK

SEQ ID NO: 41 - protein, 113 aa, synthetic construct
  REGION 1..113: note = MAGE-A1 TRAV
RGEDVEQSLFLSVREGDSSVINCTYTDSSSTYLYWYKQEPGAGLQLLTYIFSNMDMKQDQRLTVLLNKKDKHLSLRIADTQTGDSAIYFCAGSGGGTDKLIFGTGTRLQVFPN

SEQ ID NO: 42 - protein, 118 aa, synthetic construct
  REGION 1..118: note = MAGE-A1 TRBV
GAVVSQHPSWVICKSGTSVKIECRSLDFQATTMFWYRQFPKQSLMLMATSDYQTCVTYEQGVEKDKFLINHASLTLSTLTVTSAHPEDSSFYICSAREPGQGPFEQYFGPGTRLTVTE

SEQ ID NO: 43 - protein, 6 aa, synthetic construct
  REGION 1..6: note = HPV E7 TRAV CDR1
NSASQS

SEQ ID NO: 44 - protein, 6 aa, synthetic construct
  REGION 1..6: note = HPV E7 TRAV CDR2
VYSSGN

SEQ ID NO: 45 - protein, 10 aa, synthetic construct
  REGION 1..10: note = HPV E7 TRAV CDR3
AVISAGTALI

SEQ ID NO: 46 - protein, 5 aa, synthetic construct
  REGION 1..5: note = HPV E7 TRBV CDR1
SGHDT

SEQ ID NO: 47 - protein, 6 aa, synthetic construct
  REGION 1..6: note = HPV E7 TRBV CDR2
YYEEEE

SEQ ID NO: 48 - protein, 15 aa, synthetic construct
  REGION 1..15: note = HPV E7 TRBV CDR3
ASSLGWRGGLYTEAF

SEQ ID NO: 49 - protein, 109 aa, synthetic construct
  REGION 1..109: note = HPV E7 TRAV
RKEVEQDPGPFNVPEGATVAFNCTYSNSASQSFFWYRQDCRKEPKLLMSVYSSGNEDGRFTAQLNRASQYISLLIRDSKLSDSATYLCAVISAGTALIFGKGTTLSVSS

SEQ ID NO: 50 - protein, 116 aa, synthetic construct
  REGION 1..116: note = HPV E7 TRBV
DAGVTQSPTHLIKTRGQQVTLRCSPKSGHDTVSWYQQALGQGPQFIFQYYEEEERQRGNFPDRFSGHQFPNYSSELNVNALLLGDSALYLCASSLGWRGGLYTEAFFGQGTRLTVV

SEQ ID NO: 51 - protein, 6 aa, synthetic construct
  REGION 1..6: note = KRAS TRAV CDR1
YGATPY

SEQ ID NO: 52 - protein, 8 aa, synthetic construct
  REGION 1..8: note = KRAS TRAV CDR2
YFSGDTLV

SEQ ID NO: 53 - protein, 12 aa, synthetic construct
  REGION 1..12: note = KRAS TRAV CDR3
AVGVPGGYNKLI

SEQ ID NO: 54 - protein, 5 aa, synthetic construct
  REGION 1..5: note = KRAS TRBV CDR1
SGHVS

SEQ ID NO: 55 - protein, 6 aa, synthetic construct
  REGION 1..6: note = KRAS TRBV CDR2
FQNEAQ

SEQ ID NO: 56 - protein, 11 aa, synthetic construct
  REGION 1..11: note = KRAS TRBV CDR3
ASSLDRGNTIY

SEQ ID NO: 57 - protein, 114 aa, synthetic construct
  REGION 1..114: note = KRAS TRAV
AQSVTQPDIHITVSEGASLELRCNYSYGATPYLFWYVQSPGQGLQLLLKYFSGDTLVQGIKGFEAEFKRSQSSFNLRKPSVHWSDAAEYFCAVGVPGGYNKLIFGAGTRLAVHP

SEQ ID NO: 58 - protein, 113 aa, synthetic construct
  REGION 1..113: note = KRAS TRBV
GAGVSQSPRYKVAKRGQDVALRCDPISGHVSLFWYQQALGQGPEFLTYFQNEAQLDKSGLPSDRFFAERPEGSVSTLKIQRTQQEDSAVYLCASSLDRGNTIYFGEGSWLTVV

SEQ ID NO: 59 - protein, 6 aa, synthetic construct
  REGION 1..6: note = KRAS TRAV CDR1
VSGNPY

SEQ ID NO: 60 - protein, 8 aa, synthetic construct
  REGION 1..8: note = KRAS TRAV CDR2
YITGDNLV

SEQ ID NO: 61 - protein, 15 aa, synthetic construct
  REGION 1..15: note = KRAS TRAV CDR3
AVRDIEGAGNNRKLI

SEQ ID NO: 62 - protein, 5 aa, synthetic construct
  REGION 1..5: note = KRAS TRBV CDR1
SGHNS

SEQ ID NO: 63 - protein, 6 aa, synthetic construct
  REGION 1..6: note = KRAS TRBV CDR2
FNNNVP

SEQ ID NO: 64 - protein, 11 aa, synthetic construct
  REGION 1..11: note = KRAS TRBV CDR1
ASSEGFYTEAF

SEQ ID NO: 65 - protein, 117 aa, synthetic construct
  REGION 1..117: note = KRAS TRAV
AQSVAQPEDQVNVAEGNPLTVKCTYSVSGNPYLFWYVQYPNRGLQFLLKYITGDNLVKGSYGFEAEFNKSQTSFHLKKPSALVSDSALYFCAVRDIEGAGNNRKLIWGLGTSLAVNP

SEQ ID NO: 66 - protein, 113 aa, synthetic construct
  REGION 1..113: note = KRAS TRBV
DAGVIQSPRHEVTEMGQEVTLRCKPISGHNSLFWYRQTMMRGLELLIYFNNNVPIDDSGMPEDRFSAKMPNASFSTLKIQPSEPRDSAVYFCASSEGFYTEAFFGQGTRLTVV

SEQ ID NO: 67 - protein, 6 aa, synthetic construct
  REGION 1..6: note = KRAS TRAV CDR1
NSASDY

SEQ ID NO: 68 - protein, 7 aa, synthetic construct
  REGION 1..7: note = KRAS TRAV CDR2
IRSNMDK

SEQ ID NO: 69 - protein, 13 aa, synthetic construct
  REGION 1..13: note = KRAS TRAV CDR3
AENSDGTSYGKLT

SEQ ID NO: 70 - protein, 5 aa, synthetic construct
  REGION 1..5: note = KRAS TRBV CDR1
SGHAT

SEQ ID NO: 71 - protein, 6 aa, synthetic construct
  REGION 1..6: note = KRAS TRBV CDR2
FQNNGV

SEQ ID NO: 72 - protein, 13 aa, synthetic construct
  REGION 1..13: note = KRAS TRBV CDR3
ASSLVGSPDYEQY

SEQ ID NO: 73 - protein, 114 aa, synthetic construct
  REGION 1..114: note = KRAS TRAV
GESVGLHLPTLGVQEGDNSIINCAYSNSASDYFIWYKQESGKGPQFIIDIRSNMDKRQGQRVTVLLNKTVKHLSLQIAATQPGDSAVYFCAENSDGTSYGKLTFGQGTILTVHP

SEQ ID NO: 74 - protein, 115 aa, synthetic construct
  REGION 1..115: note = KRAS TRBV
EAGVAQSPRYKIIEKRQSVAFWCNPISGHATLYWYQQILGQGPKLLIQFQNNGVVDDSQLPKDRFSAERLKGVDSTLKIQPAKLEDSAVYLCASSLVGSPDYEQYFGPGTRLTVT

SEQ ID NO: 75 - protein, 6 aa, synthetic construct
  REGION 1..6: note = KRAS TRAV CDR1
DRGSQS

SEQ ID NO: 76 - protein, 6 aa, synthetic construct
  REGION 1..6: note = KRAS TRAV CDR2
IYSNGD

SEQ ID NO: 77 - protein, 12 aa, synthetic construct
  REGION 1..12: note = KRAS TRAV CDR3
AVNLGAAGNKLT

SEQ ID NO: 78 - protein, 5 aa, synthetic construct
  REGION 1..5: note = KRAS TRBV CDR1
SGHAT

SEQ ID NO: 79 - protein, 6 aa, synthetic construct
  REGION 1..6: note = KRAS TRBV CDR2
FQNNGV

SEQ ID NO: 80 - protein, 13 aa, synthetic construct
  REGION 1..13: note = KRAS TRBV CDR3
ASSFSDSYNSPLH

SEQ ID NO: 81 - protein, 112 aa, synthetic construct
  REGION 1..112: note = KRAS TRAV
QKEVEQNSGPLSVPEGAIASLNCTYSDRGSQSFFWYRQYSGKSPELIMSIYSNGDKEDGRFTAQLNKASQYVSLLIRDSQPSDSATYLCAVNLGAAGNKLTFGGGTRVLVKP

SEQ ID NO: 82 - protein, 115 aa, synthetic construct
  REGION 1..115: note = KRAS TRBV
EAGVAQSPRYKIIEKRQSVAFWCNPISGHATLYWYQQILGQGPKLLIQFQNNGVVDDSQLPKDRFSAERLKGVDSTLKIQPAKLEDSAVYLCASSFSDSYNSPLHFGNGTRLTVT

SEQ ID NO: 83 - protein, 6 aa, synthetic construct
  REGION 1..6: note = KRAS TRAV CDR1
NSASQS

SEQ ID NO: 84 - protein, 6 aa, synthetic construct
  REGION 1..6: note = KRAS TRAV CDR2
VYSSGN

SEQ ID NO: 85 - protein, 8 aa, synthetic construct
  REGION 1..8: note = KRAS TRAV CDR3
VVTNARLM

SEQ ID NO: 86 - protein, 5 aa, synthetic construct
  REGION 1..5: note = KRAS TRBV CDR1
MNHEY

SEQ ID NO: 87 - protein, 6 aa, synthetic construct
  REGION 1..6: note = KRAS TRBV CDR2
SMNVEV

SEQ ID NO: 88 - protein, 14 aa, synthetic construct
  REGION 1..14: note = KRAS TRBV CDR3
ASTSIVSSGRGEQF

SEQ ID NO: 89 - protein, 107 aa, synthetic construct
  REGION 1..107: note = KRAS TRAV
RKEVEQDPGPFNVPEGATVAFNCTYSNSASQSFFWYRQDCRKEPKLLMSVYSSGNEDGRFTAQLNRASQYISLLIRDSKLSDSATYLCVVTNARLMFGDGTQLVVKP

SEQ ID NO: 90 - protein, 115 aa, synthetic construct
  REGION 1..115: note = KRAS TRBV
EAQVTQNPRYLITVTGKKLTVTCSQNMNHEYMSWYRQDPGLGLRQIYYSMNVEVTDKGDVPEGYKVSRKEKRNFPLILESPSPNQTSLYFCASTSIVSSGRGEQFFGPGTRLTVL

SEQ ID NO: 91 - protein, 108 aa, synthetic construct
  REGION 1..108: note = gp100 TRAV
SQQGEEDPQALSIQEGENATMNCSYKTSINNLQWYRQNSGRGLVHLILIRSNEREKHSGRLRVTLDTSKKSSSLLITASRAADTASYFCATDGSTPMQFGKGTRLSVI

SEQ ID NO: 92 - protein, 112 aa, synthetic construct
  REGION 1..112: note = gp100 TRBV
DGGITQSPKYLFRKEGQNVTLSCEQNLNHDAMYWYRQDPGQGLRLIYYSWAQGDFQKGDIAEGYSVSREKKESFPLTVTSAQKNPTAFYLCASSWGAPYEQYFGPGTRLTVT

SEQ ID NO: 93 - protein, 108 aa, synthetic construct
  REGION 1..108: note = gp100 TRAV
SQQGEEDPQALSIQEGENATMNCSYKTSINNLQWYRQNSGRGLVHLILIRSNEREKHSGRLRVTLDTSKKSSSLLITASRACDTASYFCATDGSTPMQFGKGTRLSVI

SEQ ID NO: 94 - protein, 112 aa, synthetic construct
  REGION 1..112: note = gp100 TRBV
DGGITQSPKYLFRKEGQNVTLSCEQNLNHDAMYWYRQDPGQGLRLIYYSWAQGDFQKGDIAEGYSVSREKKESFPLTVTSAQKCPTAFYLCASSWGAPYEQYFGPGTRLTVT

SEQ ID NO: 95 - protein, 122 aa, synthetic construct
  REGION 1..122: note = CD3 VH
EVQLVESGGGLVQPGGSLRLSCAASGYSFTGYTMNWVRQAPGKCLEWVALINPYKGVSTYNQKFKDRFTISVDKSKNTAYLQMNSLRAEDTAVYYCARSGYYGDSDWYFDVWGQGTLVTVSS

SEQ ID NO: 96 - protein, 122 aa, synthetic construct
  REGION 1..122: note = CD3 VH
EVQLVESGGGLVQPGGSLRLSCAASGYSFTGYTMNWVRQAPGKCLEWVALINPYKGVSTYNQKFKDRFTISVDKSKNTAYLQMNSLRACDTAVYYCARSGYYGDSDWYFDVWGQGTLVTVSS

SEQ ID NO: 97 - protein, 120 aa, synthetic construct
  REGION 1..120: note = CD28 VH
QVQLVQSGAEVKKPGASVKVSCKASGYTFTSYYIHWVRQAPGQGLEWIGYIYPGNVNTNYNEKFKDRATLTVDTSISTAYMELSRLRSDDTAVYFCTRSHYGLDWNFDVWGQGTTVTVSS

SEQ ID NO: 98 - protein, 120 aa, synthetic construct
  REGION 1..120: note = CD28 VH
QVQLVQSGAEVKKPGASVKVSCKASGYTFTSYYIHWVRQAPGQGLEWIGYIYPGNVNTNYNEKFKDRATLTVDTSISTAYMELSRLRSCDTAVYFCTRSHYGLDWNFDVWGQGTTVTVSS

SEQ ID NO: 99 - protein, 121 aa, synthetic construct
  REGION 1..121: note = 4-1BB VH
EVQLLESGGGLVQPGGSLRLSCAASGFTFSSYDMSWVRQAPGKCLEWVSWISYSGGSIYYADSVKGRFTISRDNSKNTLYLQMNSLRAEDTAVYYCARDAQRNSMREFDYWGQGTLVTVSS

SEQ ID NO: 100 - protein, 117 aa, synthetic construct
  REGION 1..117: note = 4-1BB VH
EVQLVESGGGLVQPGRSLRLSCTASGFSLNDYWMSWVRQAPGKGLEWVGYIDVGGSLYYAASVKGRFTISRDDSKSIAYLQMNSLKTEDTAVYYCARGGLTYGFDLWGQGTLVTVSS

SEQ ID NO: 101 - protein, 107 aa, synthetic construct
  REGION 1..107: note = CD3 VL
DIQMTQSPSSLSASVGDRVTITCRASQDIRNYLNWYQQKPGKAPKLLIYYTSRLESGVPSRFSGSGSGTDYTLTISSLQPEDFATYYCQQGNTLPWTFGCGTKVEIK

SEQ ID NO: 102 - protein, 107 aa, synthetic construct
  REGION 1..107: note = CD3 VL
DIQMTQSPSSLSASVGDRVTITCRASQDIRNYLNWYQQKPGKAPKLLIYYTSRLESGVPSRFSGSGSGTDYTLTISSLQPCDFATYYCQQGNTLPWTFGCGTKVEIK

SEQ ID NO: 103 - protein, 107 aa, synthetic construct
  REGION 1..107: note = CD28 VL
DIQMTQSPSSLSASVGDRVTITCHASQNIYVWLNWYQQKPGKAPKLLIYKASNLHTGVPSRFSGSGSGTDFTLTISSLQPEDFATYYCQQGQTYPYTFGGGTKVEIK

SEQ ID NO: 104 - protein, 107 aa, synthetic construct
  REGION 1..107: note = CD28 VL
DIQMTQSPSSLSASVGDRVTITCHASQNIYVWLNWYQQKPGKAPKLLIYKASNLHTGVPSRFSGSGSGTDFTLTISSLQPCDFATYYCQQGQTYPYTFGGGTKVEIK

SEQ ID NO: 105 - protein, 110 aa, synthetic construct
  REGION 1..110: note = 4-1BB VL
QSVLTQPPSASGTPGQRVTISCSGSSSNIGNNYVTWYQQLPGTAPKLLIYADSHRPSGVPDRFSGSKSGTSASLAISGLRSEDEADYYCATWDYSLSGYVFGCGTKLTVL

SEQ ID NO: 106 - protein, 110 aa, synthetic construct
  REGION 1..110: note = 4-1BB VL
DIVMTQSPSSLSASVGDRVTITCQASEDISSYLAWYQQKPGKAPKRLIYGASDLASGVPSRFSASGSGTDYTFTISSLQPEDIATYYCHYYATISGLGVAFGGGTKVEIK

SEQ ID NO: 107 - protein, 113 aa, synthetic construct
  REGION 1..113: note = MAGE-A1 TRAV
RGEDVEQSLFLSVREGDSSVINCTYTDSSSTYLYWYKQEPGAGLQLLTYTWPHMDMKQDQRLTVLLNKKDKHLSLRIADTQTGDSAIYFCAGSGGGTDKLIFGTGTRLQVFPN

SEQ ID NO: 108 - protein, 118 aa, synthetic construct
  REGION 1..118: note = MAGE-A1 TRBV
GAVVSQHPSWVICKSGTSVKIECRSLDFQATTMFWYRQFPKQSLMLMATSNEGSKATYEQGVEKDKFLINHASLTLSTLTVTSAHPEDSSFYICSAREPGQGPYEQYFGPGTRLTVTE

SEQ ID NO: 109 - protein, 231 aa, synthetic construct
  REGION 1..231: note = Hinge-CH2-CH3 Hole, KiH-dS PVA-AAS N297Q T366S-L368A-Y407V Y349C
EPKSSDKTHTCPPCPAPPVAGPSVFLFPPKPKDTLMISRTPEVTCVVVDVSHEDPEVKFNWYVDGVEVHNAKTKPREEQYQSTYRVVSVLTVLHQDWLNGKEYKCKVSNKALPASIEKTISKAKGQPREPQVCTLPPSRDELTKNQVSLSCAVKGFYPSDIAVEWESNGQPENNYKTTPPVLDSDGSFFLVSKLTVDKSRWQQGNVFSCSVMHEALHNHYTQKSLSLSPGK

SEQ ID NO: 110 - protein, 231 aa, synthetic construct
  REGION 1..231: note = Hinge-CH2-CH3 Knob, KiH-dS PVA-AAS N297Q T366W S354C
EPKSSDKTHTCPPCPAPPVAGPSVFLFPPKPKDTLMISRTPEVTCVVVDVSHEDPEVKFNWYVDGVEVHNAKTKPREEQYQSTYRVVSVLTVLHQDWLNGKEYKCKVSNKALPASIEKTISKAKGQPREPQVYTLPPCRDELTKNQVSLWCLVKGFYPSDIAVEWESNGQPENNYKTTPPVLDSDGSFFLYSKLTVDKSRWQQGNVFSCSVMHEALHNHYTQKSLSLSPGK

SEQ ID NO: 111 - protein, 231 aa, synthetic construct
  REGION 1..231: note = Hinge-CH2-CH3 Hole, KiH-dS PVA-GSS N297Q T366S-L368A-Y407V Y349C
EPKSSDKTHTCPPCPAPPVAGPSVFLFPPKPKDTLMISRTPEVTCVVVDVSHEDPEVKFNWYVDGVEVHNAKTKPREEQYQSTYRVVSVLTVLHQDWLNGKEYKCKVSNKGLPSSIEKTISKAKGQPREPQVCTLPPSRDELTKNQVSLSCAVKGFYPSDIAVEWESNGQPENNYKTTPPVLDSDGSFFLVSKLTVDKSRWQQGNVFSCSVMHEALHNHYTQKSLSLSPGK

SEQ ID NO: 112 - protein, 231 aa, synthetic construct
  REGION 1..231: note = Hinge-CH2-CH3 Knob, KiH-dS PVA-GSS N297Q T366W S354C
EPKSSDKTHTCPPCPAPPVAGPSVFLFPPKPKDTLMISRTPEVTCVVVDVSHEDPEVKFNWYVDGVEVHNAKTKPREEQYQSTYRVVSVLTVLHQDWLNGKEYKCKVSNKGLPSSIEKTISKAKGQPREPQVYTLPPCRDELTKNQVSLWCLVKGFYPSDIAVEWESNGQPENNYKTTPPVLDSDGSFFLYSKLTVDKSRWQQGNVFSCSVMHEALHNHYTQKSLSLSPGK

SEQ ID NO: 113 - protein, 231 aa, synthetic construct
  REGION 1..231: note = Hinge-CH2-CH3 Hole, KiH-dS PVA-GSS T366S-L368A-Y407V Y349C
EPKSSDKTHTCPPCPAPPVAGPSVFLFPPKPKDTLMISRTPEVTCVVVDVSHEDPEVKFNWYVDGVEVHNAKTKPREEQYNSTYRVVSVLTVLHQDWLNGKEYKCKVSNKGLPSSIEKTISKAKGQPREPQVCTLPPSRDELTKNQVSLSCAVKGFYPSDIAVEWESNGQPENNYKTTPPVLDSDGSFFLVSKLTVDKSRWQQGNVFSCSVMHEALHNHYTQKSLSLSPGK

SEQ ID NO: 114 - protein, 231 aa, synthetic construct
  REGION 1..231: note = Hinge-CH2-CH3 Knob, KiH-dS PVA-GSS T366W S354C
EPKSSDKTHTCPPCPAPPVAGPSVFLFPPKPKDTLMISRTPEVTCVVVDVSHEDPEVKFNWYVDGVEVHNAKTKPREEQYNSTYRVVSVLTVLHQDWLNGKEYKCKVSNKGLPSSIEKTISKAKGQPREPQVYTLPPCRDELTKNQVSLWCLVKGFYPSDIAVEWESNGQPENNYKTTPPVLDSDGSFFLYSKLTVDKSRWQQGNVFSCSVMHEALHNHYTQKSLSLSPGK

SEQ ID NO: 115 - protein, 231 aa, synthetic construct
  REGION 1..231: note = Hinge-CH2-CH3, KiH-dS PVA-GSS
EPKSSDKTHTCPPCPAPPVAGPSVFLFPPKPKDTLMISRTPEVTCVVVDVSHEDPEVKFNWYVDGVEVHNAKTKPREEQYNSTYRVVSVLTVLHQDWLNGKEYKCKVSNKGLPSSIEKTISKAKGQPREPQVYTLPPSRDELTKNQVSLTCLVKGFYPSDIAVEWESNGQPENNYKTTPPVLDSDGSFFLYSKLTVDKSRWQQGNVFSCSVMHEALHNHYTQKSLSLSPGK

SEQ ID NO: 116 - protein, 231 aa, synthetic construct; identical to SEQ ID NO: 115
  REGION 1..231: note = Hinge-CH2-CH3, KiH-dS PVA-GSS

SEQ ID NO: 117 - protein, 231 aa, synthetic construct
  REGION 1..231: note = Hinge-CH2-CH3 FcK/O, KiH-dS PVA-GSS D356K D399K
EPKSSDKTHTCPPCPAPPVAGPSVFLFPPKPKDTLMISRTPEVTCVVVDVSHEDPEVKFNWYVDGVEVHNAKTKPREEQYNSTYRVVSVLTVLHQDWLNGKEYKCKVSNKGLPSSIEKTISKAKGQPREPQVYTLPPSRKELTKNQVSLTCLVKGFYPSDIAVEWESNGQPENNYKTTPPVLKSDGSFFLYSKLTVDKSRWQQGNVFSCSVMHEALHNHYTQKSLSLSPGK

SEQ ID NO: 118 - protein, 231 aa, synthetic construct
  REGION 1..231: note = Hinge-CH2-CH3 FcK/O, KiH-dS PVA-GSS K392D K409D
EPKSSDKTHTCPPCPAPPVAGPSVFLFPPKPKDTLMISRTPEVTCVVVDVSHEDPEVKFNWYVDGVEVHNAKTKPREEQYNSTYRVVSVLTVLHQDWLNGKEYKCKVSNKGLPSSIEKTISKAKGQPREPQVYTLPPSRDELTKNQVSLTCLVKGFYPSDIAVEWESNGQPENNYDTTPPVLDSDGSFFLYSDLTVDKSRWQQGNVFSCSVMHEALHNHYTQKSLSLSPGK

SEQ ID NO: 119 - protein, 231 aa, synthetic construct
  REGION 1..231: note = Hinge-CH2-CH3 FcK/O, KiH-dS PVA-GSS PPV-KKK
EPKSSDKTHTCPPCPAPPVAGPSVFLFPPKPKDTLMISRTPEVTCVVVDVSHEDPEVKFNWYVDGVEVHNAKTKPREEQYNSTYRVVSVLTVLHQDWLNGKEYKCKVSNKGLPSSIEKTISKAKGQPREPQVYTLPPSRDELTKNQVSLTCLVKGFYPSDIAVEWESNGQPENNYKTTKKKLDSDGSFFLYSKLTVDKSRWQQGNVFSCSVMHEALHNHYTQKSLSLSPGK

SEQ ID NO: 120 - protein, 231 aa, synthetic construct
  REGION 1..231: note = Hinge-CH2-CH3 FcK/O, KiH-dS PVA-GSS TPP-DDD
EPKSSDKTHTCPPCPAPPVAGPSVFLFPPKPKDTLMISRTPEVTCVVVDVSHEDPEVKFNWYVDGVEVHNAKTKPREEQYNSTYRVVSVLTVLHQDWLNGKEYKCKVSNKGLPSSIEKTISKAKGQPREPQVYTLPPSRDELTKNQVSLTCLVKGFYPSDIAVEWESNGQPENNYKTDDDVLDSDGSFFLYSKLTVDKSRWQQGNVFSCSVMHEALHNHYTQKSLSLSPGK

SEQ ID NO: 121 - protein, 12 aa, synthetic construct
  REGION 1..12: note = Linker
GGEGGGSEGGGS

SEQ ID NO: 122-123 - skipped (2 entries)

SEQ ID NO: 124 - protein, 21 aa, synthetic construct
  REGION 1..21: note = IgG1 Hinge region
EPKSCDKTHTCPPCPAPELLG

SEQ ID NO: 125 - protein, 19 aa, synthetic construct
  REGION 1..19: note = IgG2 Hinge region
ERKCCVECPPCPAPPVAGP

SEQ ID NO: 126 - protein, 18 aa, synthetic construct
  REGION 1..18: note = IgG4 Hinge region
ESKYGPPCPSCPAPEFLG

SEQ ID NO: 127 - protein, 104 aa, synthetic construct
  REGION 1..104: note = IgG1 CH2
GPSVFLFPPKPKDTLMISRTPEVTCVVVDVSHEDPEVKFNWYVDGVEVHNAKTKPREEQYNSTYRVVSVLTVLHQDWLNGKEYKCKVSNKALPAPIEKTISKAK

SEQ ID NO: 128 - protein, 104 aa, synthetic construct
  REGION 1..104: note = IgG2 CH2
GPSVFLFPPKPKDTLMISRTPEVTCVVVDVSHEDPEVQFNWYVDGVEVHNAKTKPREEQFNSTFRVVSVLTVVHQDWLNGKEYKCKVSNKGLPAPIEKTISKTK

SEQ ID NO: 129 - protein, 104 aa, synthetic construct
  REGION 1..104: note = IgG4 CH2
GPSVFLFPPKPKDTLMISRTPEVTCVVVDVSQEDPEVQFNWYVDGVEVHNAKTKPREEQFNSTYRVVSVLTVLHQDWLNGKEYKCKVSNKGLPSSIEKTISKAK

SEQ ID NO: 130 - protein, 107 aa, synthetic construct
  REGION 1..107: note = IgG1 CH3
GQPREPQVYTLPPSRDELTKNQVSLTCLVKGFYPSDIAVEWESNGQPENNYKTTPPVLDSDGSFFLYSKLTVDKSRWQQGNVFSCSVMHEALHNHYTQKSLSLSPGK

SEQ ID NO: 131 - protein, 107 aa, synthetic construct
  REGION 1..107: note = IgG2 CH3
GQPREPQVYTLPPSREEMTKNQVSLTCLVKGFYPSDISVEWESNGQPENNYKTTPPMLDSDGSFFLYSKLTVDKSRWQQGNVFSCSVMHEALHNHYTQKSLSLSPGK

SEQ ID NO: 132 - protein, 107 aa, synthetic construct
  REGION 1..107: note = IgG4 CH3
GQPREPQVYTLPPSQEEMTKNQVSLTCLVKGFYPSDIAVEWESNGQPENNYKTTPPVLDSDGSFFLYSRLTVDKSRWQEGNVFSCSVMHEALHNHYTQKSLSLSLGK

SEQ ID NO: 133 - protein, 21 aa, synthetic construct
  REGION 1..21: note = Hinge region
EPKSSDKTHTCPPCPAPPVAG

SEQ ID NO: 134 - protein, 15 aa, synthetic construct
  REGION 1..15: note = Hinge region
EPKSSDKTHTCPPCP

SEQ ID NO: 135 - protein, 20 aa, synthetic construct
  REGION 1..20: note = Hinge region
PKSSDKTHTCPPCPAPPVAG

SEQ ID NO: 136 - protein, 19 aa, synthetic construct
  REGION 1..19: note = Hinge region
PKSSDKTHTCPPCPAPPVA

SEQ ID NO: 137 - protein, 19 aa, synthetic construct
  REGION 1..19: note = Hinge region
KSSDKTHTCPPCPAPPVAG

SEQ ID NO: 138 - protein, 18 aa, synthetic construct
  REGION 1..18: note = Hinge region
KSSDKTHTCPPCPAPPVA

SEQ ID NO: 139 - protein, 18 aa, synthetic construct
  REGION 1..18: note = Hinge region
SSDKTHTCPPCPAPPVAG

SEQ ID NO: 140 - protein, 17 aa, synthetic construct
  REGION 1..17: note = Hinge region
SSDKTHTCPPCPAPPVA

SEQ ID NO: 141 - protein, 17 aa, synthetic construct
  REGION 1..17: note = Hinge region
SDKTHTCPPCPAPPVAG

SEQ ID NO: 142 - protein, 16 aa, synthetic construct
  REGION 1..16: note = Hinge region
SDKTHTCPPCPAPPVA

SEQ ID NO: 143 - protein, 16 aa, synthetic construct
  REGION 1..16: note = Hinge region
DKTHTCPPCPAPPVAG

SEQ ID NO: 144 - protein, 15 aa, synthetic construct
  REGION 1..15: note = Hinge region
DKTHTCPPCPAPPVA

SEQ ID NO: 145 - protein, 15 aa, synthetic construct
  REGION 1..15: note = Hinge region
KTHTCPPCPAPPVAG

SEQ ID NO: 146 - protein, 14 aa, synthetic construct
  REGION 1..14: note = Hinge region
KTHTCPPCPAPPVA

SEQ ID NO: 147 - protein, 14 aa, synthetic construct
  REGION 1..14: note = Hinge region
THTCPPCPAPPVAG

SEQ ID NO: 148 - protein, 12 aa, synthetic construct
  REGION 1..12: note = Hinge region
THTCPPCPAPPV

SEQ ID NO: 149 - protein, 13 aa, synthetic construct
  REGION 1..13: note = Hinge region
HTCPPCPAPPVAG

SEQ ID NO: 150 - protein, 12 aa, synthetic construct
  REGION 1..12: note = Hinge region
HTCPPCPAPPVA

SEQ ID NO: 151 - protein, 12 aa, synthetic construct
  REGION 1..12: note = Hinge region
TCPPCPAPPVAG

SEQ ID NO: 152 - protein, 11 aa, synthetic construct
  REGION 1..11: note = Hinge region
TCPPCPAPPVA

SEQ ID NO: 153 - protein, 11 aa, synthetic construct
  REGION 1..11: note = Hinge region
CPPCPAPPVAG

SEQ ID NO: 154 - protein, 10 aa, synthetic construct
  REGION 1..10: note = Hinge region
CPPCPAPPVA

SEQ ID NO: 155 - protein, 10 aa, synthetic construct
  REGION 1..10: note = Hinge region
PPCPAPPVAG

SEQ ID NO: 156 - protein, 9 aa, synthetic construct
  REGION 1..9: note = Hinge region
PPCPAPPVA

SEQ ID NO: 157 - protein, 8 aa, synthetic construct
  REGION 1..8: note = Hinge region
CPAPPVAG

SEQ ID NO: 158 - protein, 7 aa, synthetic construct
  REGION 1..7: note = Hinge region
CPAPPVA

SEQ ID NO: 159 - protein, 8 aa, synthetic construct
  REGION 1..8: note = Hinge region
CPAPPVAG

SEQ ID NO: 160 - protein, 6 aa, synthetic construct
  REGION 1..6: note = Hinge region
PAPPVA

SEQ ID NO: 161 - protein, 104 aa, synthetic construct
  REGION 1..104: note = CH2
GPSVFLFPPKPKDTLMISRTPEVTCVVVDVSHEDPEVKFNWYVDGVEVHNAKTKPREEQYQSTYRVVSVLTVLHQDWLNGKEYKCKVSNKALPASIEKTISKAK

SEQ ID NO: 162 - protein, 104 aa, synthetic construct
  REGION 1..104: note = CH2
GPSVFLFPPKPKDTLMISRTPEVTCVVVDVSHEDPEVKFNWYVDGVEVHNAKTKPREEQYNSTYRVVSVLTVLHQDWLNGKEYKCKVSNKALPASIEKTISKAK

SEQ ID NO: 163 - protein, 104 aa, synthetic construct
  REGION 1..104: note = CH2
GPSVFLFPPKPKDTLMISRTPEVTCVVVDVSHEDPEVKFNWYVDGVEVHNAKTKPREEQYNSTYRVVSVLTVLHQDWLNGKEYKCKVSNKGLPSSIEKTISKAK

SEQ ID NO: 164 - protein, 19 aa, synthetic construct
  REGION 1..19: note = Signal peptide
MGWSLILLFLVAVATRVHS

SEQ ID NO: 165 - protein, 9 aa, synthetic construct
  REGION 1..9: note = gp100 antigen epitope
YLEPGPVTA

SEQ ID NO: 166 - protein, 9 aa, synthetic construct
  REGION 1..9: note = gp100 antigen epitope variant
YLEPGPVTV